European Patent Application EP 4 424 299 A1, published September 4, 2024. Title: Cosmetic composition for the prevention or improvement of inflammatory skin diseases comprising a strain of the genus Cutibacterium. Applicant: CJ CheilJedang Corporation. The sequence listing filed with the application follows.

SEQUENCE LISTING (8 sequences)

SEQ ID NO: 1 - DNA, 20 bp, synthetic construct
  misc_feature 1..20: note = synthetic_27F primer
  source 1..20: mol_type = other DNA
agagtttgatcmtggctcag

SEQ ID NO: 2 - DNA, 22 bp, synthetic construct
  misc_feature 1..22: note = synthetic_1482R primer
  source 1..22: mol_type = other DNA
tacggytaccttgttacgactt

SEQ ID NO: 3 - DNA, 19 bp, synthetic construct
  misc_feature 1..19: note = synthetic_515F primer
  source 1..19: mol_type = other DNA
gtgccagcmgccgcggtaa

SEQ ID NO: 4 - DNA, 20 bp, synthetic construct
  misc_feature 1..20: note = synthetic_518F primer
  source 1..20: mol_type = other DNA
ccagcagccgcggtaatacg

SEQ ID NO: 5 - DNA, 22 bp, synthetic construct
  misc_feature 1..22: note = synthetic_recA_F primer
  source 1..22: mol_type = other DNA
agctcggtggggttctctcatc

SEQ ID NO: 6 - DNA, 23 bp, synthetic construct
  misc_feature 1..23: note = synthetic_recA_R primer
  source 1..23: mol_type = other DNA
gcttcctcataccactggtcatc

SEQ ID NO: 7 - DNA, 22 bp, synthetic construct
  misc_feature 1..22: note = synthetic_recA_F primer
  source 1..22: mol_type = other DNA
ggtaccactgccatcttcatta

SEQ ID NO: 8 - DNA, 1525 bp, synthetic construct
  misc_feature 1..1525: note = synthetic_16S rRNA gene sequence of Cutibacterium acnesCJRS-10651, CJRS-10652, CJRS-10653, CJRS-10654, CJRS-10655, andCJRS-10656
  source 1..1525: mol_type = other DNA
tcattggagagtttgatcctggctcaggacgaacgctggcggcgtgcttaacacatgcaagtcgaacggaaaggccctgcttttgtggggtgctcgagtggcgaacgggtgagtaacacgtgagtaacctgcccttgactttgggataacttcaggaaactggggctaataccggataggagctcctgctgcatggtgggggttggaaagtttcggcggttggggatggactcgcggcttatcagcttgttggtggggtagtggcttaccaaggctttgacgggtagccggcctgagagggtgaccggccacattgggactgagatacggcccagactcctacgggaggcagcagtggggaatattgcacaatgggcggaagcctgatgcagcaacgccgcgtgcgggatgacggccttcgggttgtaaaccgctttcgcctgtgacgaagcgtgagtgacggtaatgggtaaagaagcaccggctaactacgtgccagcagccgcggtgatacgtagggtgcgagcgttgtccggatttattgggcgtaaagggctcgtaggtggttgatcgcgtcggaagtgtaatcttggggcttaaccctgagcgtgctttcgatacgggttgacttgaggaaggtaggggagaatggaattcctggtggagcggtggaatgcgcagatatcaggaggaacaccagtggcgaaggcggttctctgggcctttcctgacgctgaggagcgaaagcgtggggagcgaacaggcttagataccctggtagtccacgctgtaaacggtgggtactaggtgtggggtccattccacgggttccgcgccgtagctaacgctttaagtaccccgcctggggagtacggccgcaaggctaaaactcaaaggaattgacggggccccgcacaagcggcggagcatgcggattaattcgatgcaacgcgtagaaccttacctgggtttgacatggatcgggagtgctcagagatgggtgtgcctcttttggggtcggttcacaggtggtgcatggctgtcgtcagctcgtgtcgtgagatgttgggttaagtcccgcaacgagcgcaacccttgttcactgttgccagcacgttatggtggggactcagtggagaccgccggggtcaactcggaggaaggtggggatgacgtcaagtcatcatgccccttatgtccagggcttcacgcatgctacaatggctggtacagagagtggcgagcctgtgagggtgagcgaatctcggaaagccggtctcagttcggattggggtctgcaactcgacctcatgaagtcggagtcgctagtaatcgcagatcagcaacgctgcggtgaatacgttcccggggcttgtacacaccgcccgtcaagtcatgaaagttggtaacacccgaagccggtggcctaaccgttgtgggggagccgtcgaaggtgggactggtgattaggactaagtcgtaacaaggtagccgtaccggaaggtgcggctggatcacctccttt